European Patent Specification EP 3 793 573 B1, published October 23, 2024. Title: SUBSETS OF HUMAN NATURAL KILLER CELLS WITH ENHANCED ANTIBODY-DIRECTED IMMUNE RESPONSES. Applicant: Indapta Therapeutics, Inc. DIPIERRO, Guy DOS SANTOS, Gary. Application Not Yet Assigned. The sequence listing filed with the application follows.

SEQUENCE LISTING (12 sequences)

SEQ ID NO: 1 - DNA, 21 bp, artificial sequence
  158V Primer
atatttacagaatggcacagg

SEQ ID NO: 2 - DNA, 20 bp, artificial sequence
  158V Primer
gacttggtacccaggttgaa

SEQ ID NO: 3 - DNA, 32 bp, artificial sequence
  158V Primer
atcagattcgatcctacttctgcagggggcat

SEQ ID NO: 4 - DNA, 32 bp, artificial sequence
  158V Primer
acgtgctgagcttgagtgatggtgatgttcac

SEQ ID NO: 5 - DNA, 24 bp, artificial sequence
  158V Primer
cccaactcaacttcccagtgtgat

SEQ ID NO: 6 - DNA, 30 bp, artificial sequence
  158V Primer
gaaatctaccttttcctctaatagggcaat

SEQ ID NO: 7 - DNA, 29 bp, artificial sequence
  158V Primer
gaaatctaccttttcctctaatagggcaa

SEQ ID NO: 8 - DNA, 28 bp, artificial sequence
  158V Primer
gaaatctaccttttcctctaatagggca

SEQ ID NO: 9 - protein, 238 aa, artificial sequence
  CD16 (F158)
GMRTEDLPKAVVFLEPQWYRVLEKDSVTLKCQGAYSPEDNSTQWFHNESLISSQASSYFIDAATVDDSGEYRCQTNLSTLSDPVQLEVHIGWLLLQAPRWVFKEEDPIHLRCHSWKNTALHKVTYLQNGKGRKYFHHNSDFYIPKATLKDSGSYFCRGLFGSKNVSSETVNITITQGLAVSTISSFFPPGYQVSFCLVMVLLFAVDTGLYFSVKTNIRSSTRDWKDHKFKWRKDPQDK

SEQ ID NO: 10 - protein, 16 aa, artificial sequence
  Signal peptide
MWQLLLPTALLLLVSA

SEQ ID NO: 11 - protein, 238 aa, artificial sequence
  CD16 (158V+)
GMRTEDLPKAVVFLEPQWYRVLEKDSVTLKCQGAYSPEDNSTQWFHNESLISSQASSYFIDAATVDDSGEYRCQTNLSTLSDPVQLEVHIGWLLLQAPRWVFKEEDPIHLRCHSWKNTALHKVTYLQNGKGRKYFHHNSDFYIPKATLKDSGSYFCRGLVGSKNVSSETVNITITQGLAVSTISSFFPPGYQVSFCLVMVLLFAVDTGLYFSVKTNIRSSTRDWKDHKFKWRKDPQDK

SEQ ID NO: 12 - protein, 86 aa, artificial sequence
  FcRgamma chain
MIPAVVLLLLLLVEQAAALGEPQLCYILDAILFLYGIVLTLLYCRLKIQVRKAAITSYEKSDGVYTGLSTRNQETYETLKHEKPPQ